European Patent Specification EP 3 513 799 B1, published July 9, 2025. Title: A composition comprising lactic acid bacterium as an effective ingredient for preventing or improving aggravation of skin condition caused by abnormal proliferation of specific bacterium. Applicant: Kirin Company, Limited. The sequence listing filed with the application follows.

SEQUENCE LISTING (10 sequences)

SEQ ID NO: 1 - DNA, 18 bp, Artificial
  primer
aacgaccccttcattgac

SEQ ID NO: 2 - DNA, 19 bp, Artificial
  primer
tccacgacatactcagcac

SEQ ID NO: 3 - DNA, 20 bp, Artificial
  primer
ggaaatcaccatgccctcta

SEQ ID NO: 4 - DNA, 20 bp, Artificial
  primer
gctgtctttgtgagatgcca

SEQ ID NO: 5 - DNA, 20 bp, Artificial
  primer
ccagatggagccaggtgttg

SEQ ID NO: 6 - DNA, 22 bp, Artificial
  primer
agctggagcggagacagaatcc

SEQ ID NO: 7 - DNA, 21 bp, Artificial
  primer
gcattggcaacactcgtcaga

SEQ ID NO: 8 - DNA, 20 bp, Artificial
  primer
cgggatcttggtcttctcta

SEQ ID NO: 9 - DNA, 20 bp, Artificial
  primer
tcttgttcttggtgcctgct

SEQ ID NO: 10 - DNA, 22 bp, Artificial
  primer
cgaccgctattagaacatcgac